European Patent Application EP 4 544 911 A1, published April 30, 2025. Title: INSECT NEUROPEPTIDES 9. Applicant: SOLASTA Bio Limited. The sequence listing filed with the application follows.

SEQUENCE LISTING (19 sequences)

SEQ ID NO: 1 - protein, 8 aa, synthetic construct
  source 1..8: note = ZA1 peptide
QLTFSPDW

SEQ ID NO: 2 - protein, 7 aa, synthetic construct
  source 1..7: note = ZA2 peptide
LTFSPDW

SEQ ID NO: 3 - protein, 19 aa, synthetic construct
  source 1..19: note = ZP1 peptide
LRQLQSNGEPAYRVRTPRL

SEQ ID NO: 4 - protein, 8 aa, synthetic construct
  source 1..8: note = ZP2 peptide
SVPFKPRL

SEQ ID NO: 5 - protein, 8 aa, synthetic construct
  source 1..8: note = SB-P-39
  MOD_RES 1: note = palmitoyl-glutamine
  MOD_RES 8: note = tryptophanamide
QLTFSPDW

SEQ ID NO: 6 - protein, 7 aa, synthetic construct
  source 1..7: note = SB-P-42
  MOD_RES 1: note = pyroglutamyl-leucine
  MOD_RES 7: note = tryptophanamide
LTFSPDW

SEQ ID NO: 7 - protein, 8 aa, synthetic construct
  source 1..8: note = SB-P-49
  MOD_RES 8: note = leucinamide
SVPFKPRL

SEQ ID NO: 8 - protein, 19 aa, synthetic construct
  source 1..19: note = SB-P-51
  MOD_RES 19: note = leucinamide
LRQLQSNGEPAYRVRTPRL

SEQ ID NO: 9 - protein, 12 aa, synthetic construct
  source 1..12: note = SB-P-46
  MOD_RES 12: note = leucinamide
SPPYSPPFSPRL

SEQ ID NO: 10 - protein, 11 aa, synthetic construct
  source 1..11: note = SB-P-47
  MOD_RES 11: note = leucinamide
  MOD_RES 1: note = pyroglutamyl-alanine
AIMARPQVPRL

SEQ ID NO: 11 - protein, 16 aa, synthetic construct
  source 1..16: note = SB-P-80
  MOD_RES 16: note = leucinamide
NADEDQQQSVDFTPRL

SEQ ID NO: 12 - protein, 10 aa, synthetic construct
  source 1..10: note = SB-P-81
  MOD_RES 10: note = leucinamide
GGSMTFSPRL

SEQ ID NO: 13 - protein, 8 aa, synthetic construct
  source 1..8: note = SB-P-70
  MOD_RES 8: note = glycinamide
KVKFSAWG

SEQ ID NO: 14 - protein, 10 aa, synthetic construct
  source 1..10: note = SB-P-65
  MOD_RES 10: note = glycinamide
RQKTVFSSWG

SEQ ID NO: 15 - protein, 7 aa, synthetic construct
  source 1..7: note = SB-P-66
  MOD_RES 7: note = glycinamide
PAFSSWG

SEQ ID NO: 16 - protein, 6 aa, synthetic construct
  source 1..6: note = SB-P-69
  MOD_RES 6: note = glycinamide
NFSPWG

SEQ ID NO: 17 - protein, 9 aa, synthetic construct
  source 1..9: note = SB-P-86
  MOD_RES 9: note = glycinamide
  MOD_RES 1: note = pyroglutamyl-leucine
LTFTSSWGG

SEQ ID NO: 18 - protein, 19 aa, synthetic construct
  source 1..19: note = SB-P-48
  MOD_RES 19: note = leucinamide
EQNVQSNGEPAYRVRTPRL

SEQ ID NO: 19 - protein, 8 aa, unidentified
  source 1..8: note = SB-P-41
  MOD_RES 8: note = tryptophanamide
QLTFSPDW